European Patent Specification EP 3 800 257 B1, published May 1, 2024. Title: Pan-Genotypic Agents Against Influenza Virus and Methods of Using the Same. Applicant: THE BOARD OF TRUSTEES OF THE LELAND STANFORD JUNIOR UNIVERSITY. Application PCT/US17/20241. The sequence listing filed with the application follows.

SEQUENCE LISTING (97 sequences)

SEQ ID NO: 1 - RNA, 196 nt, Artificial Sequence
  Synthetic polynucleotide
aguagaaacaaggucguuuuuaaacuauucgacacuaauugauggccauccgaauucuuuuggucgcugucuggcugucaguaaguaugcuagagucccguuuucguuucauuaccaacaccacgucuccuugcccaauuagcacauuagccuuuuuuauucuuuccauauugaauauaauugaccugcuuucgcu

SEQ ID NO: 2 - RNA, 182 nt, Artificial Sequence
  Synthetic polynucleotide
aguagaaacaaggucguuuuuaaacuauucgacacuaauugaucgccauccgaauucuuuuggucgcugucuggcugucaguaaguaugcuagagucccguuuucguuucgcgagacugcgacauuagauuucuuaguucuuuuauucuuuccauauugaauauaauugaccugcuuucgcu

SEQ ID NO: 3 - RNA, 197 nt, Artificial Sequence
  Synthetic polynucleotide
aguagaaacaggucguuuuuaaacuauucgacacuaauugauggccauccgaauucuuuuggucgcugucuggcugucuguaaguaugcuagagucccguuuucguuucggacucucaaaaacgugcgagacugcgacauuagauuucuuaguucuuuuauucuuuccauauugaauauaauugaccugcuuucgcu

SEQ ID NO: 4 - RNA, 158 nt, Artificial Sequence
  Synthetic polynucleotide
aguagaaacaaggucguuuuuaaacuauucgacacuaauugaugauggccauccgaauucuuuuggucgcugucuggcugucaguaaguaugcuagagucccguuuccguuucauuaccaacaccacgucucuugaauauaauugaccugcuuucgcu

SEQ ID NO: 5 - RNA, 178 nt, Artificial Sequence
  Synthetic polynucleotide
aguagaaacaaggucguuuuuaaauaauucgacacuaauugauggccauccgaauucuuuuggucgcugucuggcugucaguaaguaugcuagagucccguuuucguuucauuaccaacaccacgucuccuugcccuuuuauucucuccauauugaauauauuugaccugcuuucgcu

SEQ ID NO: 6 - RNA, 289 nt, Artificial Sequence
  Synthetic polynucleotide
aguagaaacaaggucguuuuuaaacuauucgacacuaauugauggccauccgaauucuuuuggucgcugucuggcugucaguaaguaugcuagagucccguuuucguuucauuaccaacacuacguccccuugcccaauuagcacauuagccuucucuccuuuugcaagauugcucaguucauugaugcuaaugcugggccauaucucuugucuucuuugcccaaaaugagaaauccucucaggacagcauauucucuccauauugaauauaauugaccugcuuucgcu

SEQ ID NO: 7 - RNA, 177 nt, Artificial Sequence
  Synthetic polynucleotide
aguagaaacaaggucguuuuuaaacuauucgacacuaauugauggccauccgaauucuuuuggucgcugucuggcugucaguaaguaugcuagagucccguuucguuucauuaccaacaccacgucuccuugcccuuuuauucuuuccauauugaauauaauugaccugcuuucgcu

SEQ ID NO: 8 - RNA, 197 nt, Artificial Sequence
  Synthetic polynucleotide
aguagaaacaaggucguuuuuaaacuauucgacacuaauugauggccauccgaauucuuuuggucgcugucuggcugucaguuaauaugcuagagucccguuuucguuucauuaccaacaccacgucuccuugcccaauuagcacgucgauagguuuuuuauucuuuccauauugaauauaaugaccugcuuucgcu

SEQ ID NO: 9 - RNA, 198 nt, Artificial Sequence
  Synthetic polynucleotide
aguagaaacaaggucguuuuuaaacuauucgacacuaauugauggccauccgaauucuuuuggucgcugucuggcugucuguaaguaugcuagagucccguuuucguuucggacucucaaaaacgugcgagacugcgacauuagauuucuuaguucuuuuauucuuuccauauugaauauaauugaccugcuuucgcu

SEQ ID NO: 10 - RNA, 178 nt, Artificial Sequence
  Synthetic polynucleotide
aguagaaacaaggucguuuuuaaacuauucgacaucuaauugauggccauccgaauucuuuuggucgcugucuggcugucaguaaguaugcuagagucccguuuucguuugacugcgacauuagauuucuuaguucuuuuauucuuuccauauugaauauaauugaccugcuuucgcu

SEQ ID NO: 11 - RNA, 182 nt, Artificial Sequence; identical to SEQ ID NO: 2
  Synthetic polynucleotide

SEQ ID NO: 12 - RNA, 59 nt, Artificial Sequence
  Synthetic polynucleotide
cgacacuaauugauggccauccgaauucuuuuggucgcugucuggcugucaguaaguau

SEQ ID NO: 13 - RNA, 59 nt, Artificial Sequence; identical to SEQ ID NO: 12
  Synthetic polynucleotide

SEQ ID NO: 14 - DNA, 108 bp, Artificial Sequence
  Synthetic polynucleotide
attgggcaaggagacgtggtgttggtaatgaaacggaaacggaactctagcatacttactgacagccagacagcgaccaaaagaattcggatggccatcaattagtgt

SEQ ID NO: 15 - DNA, 108 bp, Artificial Sequence
  Synthetic polynucleotide
attgggcaaggagacgtcgtgttggtaatgaaacggaaacggaactctagcatattaacagacagccaaacagcgacgaaaagaattcggatggcgatcaattgatgt

SEQ ID NO: 16 - DNA, 23 bp, Artificial Sequence
  Synthetic polynucleotide
tacttactgacagtcagacagcg

SEQ ID NO: 17 - DNA, 23 bp, Artificial Sequence
  Synthetic polynucleotide
cgctgtctgactgtcagtaagta

SEQ ID NO: 18 - DNA, 23 bp, Artificial Sequence
  Synthetic polynucleotide
tacttactgactcgcagacagcg

SEQ ID NO: 19 - DNA, 23 bp, Artificial Sequence
  Synthetic polynucleotide
cgctgtctgcgagtcagtaagta

SEQ ID NO: 20 - DNA, 30 bp, Artificial Sequence
  Synthetic polynucleotide
tgacagccagactgcgaccaaaagaattcg

SEQ ID NO: 21 - DNA, 30 bp, Artificial Sequence
  Synthetic polynucleotide
cgaattcttttggtcgcagtctggctgtca

SEQ ID NO: 22 - DNA, 24 bp, Artificial Sequence
  Synthetic polynucleotide
agcgaccaaaagcattcggatggc

SEQ ID NO: 23 - DNA, 24 bp, Artificial Sequence
  Synthetic polynucleotide
gccatccgaatgcttttggtcgct

SEQ ID NO: 24 - RNA, 175 nt, Artificial Sequence
  Synthetic polynucleotide
aguagaaacaaggucguuuuuaaacuauucgacacuaauugauggccauccgaauucuuuuggucgcugucggcugucaguaaguaugcuagagucccguuuucguuucauuaccaacacgacgucuccuugcuuuuauucuuuccauauugaauauaauugaccugcuuucgcu

SEQ ID NO: 25 - RNA, 151 nt, Artificial Sequence
  Synthetic polynucleotide
aguagaaacaaggucguuuuuaaacuauucgacacuaauugauggccauccgaauucuuuucgucgcugucuggcugucaguaaguaugcuagagucccguuuucguuucuuuauucuuuccauauugaauauaauugaccugcuuucgcu

SEQ ID NO: 26 - RNA, 148 nt, Artificial Sequence
  Synthetic polynucleotide
agugaaacaaggucguuuuuaaacuauucgacacuaauugauggccauccgaauucuuuuggucgcuguuuggcugucaguaaguaugcuagagucccguuuuaguuuuuauucuuuccauauugaauauaauugaccugcuuucgcu

SEQ ID NO: 27 - RNA, 59 nt, Artificial Sequence; identical to SEQ ID NO: 12
  Synthetic polynucleotide

SEQ ID NO: 28 - DNA, 29 bp, Artificial Sequence
  Synthetic polynucleotide
agaattcggatgcccatcaattagtgtcg

SEQ ID NO: 29 - DNA, 29 bp, Artificial Sequence
  Synthetic polynucleotide
cgacactaattgatgggcatccgaattct

SEQ ID NO: 30 - DNA, 23 bp, Artificial Sequence
  Synthetic polynucleotide
tacttactgacaggcagacagcg

SEQ ID NO: 31 - DNA, 23 bp, Artificial Sequence
  Synthetic polynucleotide
cgctgtctgcctgtcagtaagta

SEQ ID NO: 32 - DNA, 25 bp, Artificial Sequence
  Synthetic polynucleotide
ttcggatgggcatcaattagtgtcg

SEQ ID NO: 33 - DNA, 25 bp, Artificial Sequence
  Synthetic polynucleotide
cgacactaattgatgcccatccgaa

SEQ ID NO: 34 - DNA, 24 bp, Artificial Sequence
  Synthetic polynucleotide
atacttactgacacccagacagcg

SEQ ID NO: 35 - DNA, 24 bp, Artificial Sequence
  Synthetic polynucleotide
cgctgtctgggtgtcagtaagtat

SEQ ID NO: 36 - DNA, 24 bp, Artificial Sequence
  Synthetic polynucleotide
tcggatggccatgaattagtgtcg

SEQ ID NO: 37 - DNA, 24 bp, Artificial Sequence
  Synthetic polynucleotide
cgacactaattcatggccatccga

SEQ ID NO: 38 - DNA, 26 bp, Artificial Sequence
  Synthetic polynucleotide
agcatacttactcacagccagacagc

SEQ ID NO: 39 - DNA, 26 bp, Artificial Sequence
  Synthetic polynucleotide
gctgtctggctgtgagtaagtatgct

SEQ ID NO: 40 - DNA, 34 bp, Artificial Sequence
  Synthetic polynucleotide
ccaaaagaattaggatggccatcaattagtgtcg

SEQ ID NO: 41 - DNA, 34 bp, Artificial Sequence
  Synthetic polynucleotide
cgacactaattgatggccatcctaattcttttgg

SEQ ID NO: 42 - DNA, 29 bp, Artificial Sequence
  Synthetic polynucleotide
gacagccagacagctaccaaaagaattcg

SEQ ID NO: 43 - DNA, 29 bp, Artificial Sequence
  Synthetic polynucleotide
cgaattcttttggtagctgtctggctgtc

SEQ ID NO: 44 - RNA, 71 nt, Artificial Sequence
  Synthetic polynucleotide
ucgacacuaauugauggccauccgaauucuuuuggucgcugucuggcugucaguaaguaugcuagccuugc

SEQ ID NO: 45 - DNA, 11 bp, Artificial Sequence
  Synthetic polynucleotide
accaaaagaat

SEQ ID NO: 46 - DNA, 11 bp, Artificial Sequence
  Synthetic polynucleotide
tggccatcaat

SEQ ID NO: 47 - DNA, 11 bp, Artificial Sequence
  Synthetic polynucleotide
tagcatactta

SEQ ID NO: 48 - DNA, 8 bp, Artificial Sequence
  Synthetic polynucleotide
ccaaaaga

SEQ ID NO: 49 - DNA, 8 bp, Artificial Sequence
  Synthetic polynucleotide
catactta

SEQ ID NO: 50 - DNA, 15 bp, Artificial Sequence
  Synthetic polynucleotide
cagacacgaccaaaa

SEQ ID NO: 51 - DNA, 15 bp, Artificial Sequence
  Synthetic polynucleotide
tacttactgacagcc

SEQ ID NO: 52 - DNA, 15 bp, Artificial Sequence
  Synthetic polynucleotide
agacacgaccaaaag

SEQ ID NO: 53 - DNA, 11 bp, Artificial Sequence
  Synthetic polynucleotide
accaaaagaat

SEQ ID NO: 54 - DNA, 11 bp, Artificial Sequence
  Synthetic polynucleotide
tggccatcaat

SEQ ID NO: 55 - DNA, 11 bp, Artificial Sequence
  Synthetic polynucleotide
tagcatactta

SEQ ID NO: 56 - DNA, 15 bp, Artificial Sequence
  Synthetic polynucleotide
cgaccaaaagaattc

SEQ ID NO: 57 - DNA, 15 bp, Artificial Sequence
  Synthetic polynucleotide
cgaccaaaagaattc

SEQ ID NO: 58 - DNA, 15 bp, Artificial Sequence
  Synthetic polynucleotide
gatggccatcaatta

SEQ ID NO: 59 - DNA, 15 bp, Artificial Sequence
  Synthetic polynucleotide
gatggccatcaatta

SEQ ID NO: 60 - DNA, 15 bp, Artificial Sequence
  Synthetic polynucleotide
tctagcatacttact

SEQ ID NO: 61 - DNA, 15 bp, Artificial Sequence
  Synthetic polynucleotide
tctagcatacttact

SEQ ID NO: 62 - DNA, 15 bp, Artificial Sequence
  Synthetic polynucleotide
gaattcggatggcca

SEQ ID NO: 63 - DNA, 15 bp, Artificial Sequence
  Synthetic polynucleotide
ggccatcaattagtg

SEQ ID NO: 64 - DNA, 15 bp, Artificial Sequence
  Synthetic polynucleotide
ttcggatggccatca

SEQ ID NO: 65 - DNA, 13 bp, Artificial Sequence
  Synthetic polynucleotide
agccagacagcga

SEQ ID NO: 66 - DNA, 15 bp, Artificial Sequence
  Synthetic polynucleotide
gacagccagacagca

SEQ ID NO: 67 - DNA, 11 bp, Artificial Sequence
  Synthetic polynucleotide
  misc_feature (1)..(1): LNA
  misc_feature (4)..(4): LNA
  misc_feature (7)..(8): LNA
  misc_feature (11)..(11): LNA
accaaaagaat

SEQ ID NO: 68 - DNA, 11 bp, Artificial Sequence
  Synthetic polynucleotide
  misc_feature (1)..(1): LNA
  misc_feature (4)..(4): LNA
  misc_feature (6)..(7): LNA
  misc_feature (11)..(11): LNA
tggccatcaat

SEQ ID NO: 69 - DNA, 11 bp, Artificial Sequence
  Synthetic polynucleotide
  misc_feature (1)..(1): LNA
  misc_feature (4)..(5): LNA
  misc_feature (7)..(7): LNA
  misc_feature (11)..(11): LNA
tagcatactta

SEQ ID NO: 70 - DNA, 8 bp, Artificial Sequence
  Synthetic polynucleotide
  misc_feature (1)..(8): LNA
ccaaaaga

SEQ ID NO: 71 - DNA, 8 bp, Artificial Sequence
  Synthetic polynucleotide
  misc_feature (1)..(8): LNA
catactta

SEQ ID NO: 72 - DNA, 15 bp, Artificial Sequence
  Synthetic polynucleotide
  misc_feature (1)..(1): LNA
  misc_feature (5)..(5): LNA
  misc_feature (7)..(8): LNA
  misc_feature (10)..(11): LNA
  misc_feature (14)..(15): LNA
cagacacgaccaaaa

SEQ ID NO: 73 - DNA, 15 bp, Artificial Sequence
  Synthetic polynucleotide
  misc_feature (1)..(2): LNA
  misc_feature (4)..(4): LNA
  misc_feature (7)..(8): LNA
  misc_feature (11)..(11): LNA
  misc_feature (14)..(15): LNA
tacttactgacagcc

SEQ ID NO: 74 - DNA, 15 bp, Artificial Sequence
  Synthetic polynucleotide
  misc_feature (1)..(4): LNA
  misc_feature (12)..(15): LNA
agacacgaccaaaag

SEQ ID NO: 75 - DNA, 15 bp, Artificial Sequence
  Synthetic polynucleotide
  misc_feature (1)..(4): LNA
  misc_feature (13)..(15): LNA
tacttactgacagcc

SEQ ID NO: 76 - DNA, 15 bp, Artificial Sequence
  Synthetic polynucleotide
  misc_feature (1)..(3): LNA
  misc_feature (12)..(15): LNA
tacttactgacagcc

SEQ ID NO: 77 - DNA, 11 bp, Artificial Sequence
  Synthetic polynucleotide
  misc_feature (1)..(3): LNA
  misc_feature (9)..(11): LNA
accaaaagaat

SEQ ID NO: 78 - DNA, 11 bp, Artificial Sequence
  Synthetic polynucleotide
  misc_feature (1)..(3): LNA
  misc_feature (9)..(11): LNA
tggccatcaat

SEQ ID NO: 79 - DNA, 11 bp, Artificial Sequence
  Synthetic polynucleotide
  misc_feature (1)..(3): LNA
  misc_feature (9)..(11): LNA
tagcatactta

SEQ ID NO: 80 - DNA, 15 bp, Artificial Sequence
  Synthetic polynucleotide
  misc_feature (1)..(1): LNA
  misc_feature (5)..(6): LNA
  misc_feature (9)..(10): LNA
  misc_feature (15)..(15): LNA
cgaccaaaagaattc

SEQ ID NO: 81 - DNA, 15 bp, Artificial Sequence
  Synthetic polynucleotide
  misc_feature (1)..(4): LNA
  misc_feature (12)..(15): LNA
cgaccaaaagaattc

SEQ ID NO: 82 - DNA, 15 bp, Artificial Sequence
  Synthetic polynucleotide
  misc_feature (1)..(1): LNA
  misc_feature (3)..(4): LNA
  misc_feature (6)..(6): LNA
  misc_feature (8)..(9): LNA
  misc_feature (12)..(12): LNA
  misc_feature (15)..(15): LNA
gatggccatcaatta

SEQ ID NO: 83 - DNA, 15 bp, Artificial Sequence
  Synthetic polynucleotide
  misc_feature (1)..(4): LNA
  misc_feature (12)..(15): LNA
gatggccatcaatta

SEQ ID NO: 84 - DNA, 15 bp, Artificial Sequence
  Synthetic polynucleotide
  misc_feature (1)..(1): LNA
  misc_feature (3)..(4): LNA
  misc_feature (6)..(6): LNA
  misc_feature (8)..(9): LNA
  misc_feature (12)..(12): LNA
  misc_feature (15)..(15): LNA
tctagcatacttact

SEQ ID NO: 85 - DNA, 15 bp, Artificial Sequence
  Synthetic polynucleotide
  misc_feature (1)..(4): LNA
  misc_feature (12)..(15): LNA
tctagcatacttact

SEQ ID NO: 86 - DNA, 15 bp, Artificial Sequence
  Synthetic polynucleotide
  misc_feature (1)..(3): LNA
  misc_feature (12)..(15): LNA
gaattcggatggcca

SEQ ID NO: 87 - DNA, 15 bp, Artificial Sequence
  Synthetic polynucleotide
  misc_feature (1)..(4): LNA
  misc_feature (13)..(15): LNA
ggccatcaattagtg

SEQ ID NO: 88 - DNA, 15 bp, Artificial Sequence
  Synthetic polynucleotide
  misc_feature (1)..(4): LNA
  misc_feature (13)..(15): LNA
ttcggatggccatca

SEQ ID NO: 89 - DNA, 13 bp, Artificial Sequence
  Synthetic polynucleotide
  misc_feature (1)..(4): LNA
  misc_feature (13)..(5): LNA
agccagacagcga

SEQ ID NO: 90 - DNA, 15 bp, Artificial Sequence
  Synthetic polynucleotide
  misc_feature (1)..(4): LNA
  misc_feature (13)..(15): LNA
gacagccagacagca

SEQ ID NO: 91 - DNA, 15 bp, Artificial Sequence
  Synthetic polynucleotide
tacttactgacagtc

SEQ ID NO: 92 - DNA, 15 bp, Artificial Sequence
  Synthetic polynucleotide
tacttaccgacagcc

SEQ ID NO: 93 - DNA, 16 bp, Artificial Sequence
  Synthetic polynucleotide
ggatttcggatggcca

SEQ ID NO: 94 - DNA, 15 bp, Artificial Sequence
  Synthetic polynucleotide
  misc_feature (1)..(4): LNA
  misc_feature (13)..(15): LNA
tacttactgacagtc

SEQ ID NO: 95 - DNA, 15 bp, Artificial Sequence
  Synthetic polynucleotide
  misc_feature (1)..(4): LNA
  misc_feature (13)..(15): LNA
tacttaccgacagcc

SEQ ID NO: 96 - DNA, 16 bp, Artificial Sequence
  Synthetic polynucleotide
  misc_feature (1)..(4): LNA
  misc_feature (14)..(16): LNA
ggatttcggatggcca

SEQ ID NO: 97 - DNA, 26 bp, Artificial Sequence
  Synthetic polynucleotide
agggctcttcggccagcraaagcagg